European Patent Specification EP 3 429 609 B1, published March 1, 2023. Title: COMPOSITIONS AND METHODS FOR TREATMENT OF TYPE VII COLLAGEN DEFICIENCIES. Applicant: INTREXON CORPORATION. The sequence listing filed with the application follows.

SEQUENCE LISTING (34 sequences)

SEQ ID NO: 1 - DNA, 9169 bp, Homo sapiens
gatgacgctgcggcttctggtggccgcgctctgcgccgggatcctggcagaggcgccccgagtgcgagcccagcacagggagagagtgacctgcacgcgcctttacgccgctgacattgtgttcttactggatggctcctcatccattggccgcagcaatttccgcgaggtccgcagctttctcgaagggctggtgctgcctttctctggagcagccagtgcacagggtgtgcgctttgccacagtgcagtacagcgatgacccacggacagagttcggcctggatgcacttggctctgggggtgatgtgatccgcgccatccgtgagcttagctacaaggggggcaacactcgcacaggggctgcaattctccatgtggctgaccatgtcttcctgccccagctggcccgacctggtgtccccaaggtctgcatcctgatcacagacgggaagtcccaggacctggtggacacagctgcccaaaggctgaaggggcagggggtcaagctatttgctgtggggatcaagaatgctgaccctgaggagctgaagcgagttgcctcacagcccaccagtgacttcttcttcttcgtcaatgacttcagcatcttgaggacactactgcccctcgtttcccggagagtgtgcacgactgctggtggcgtgcctgtgacccgacctccggatgactcgacctctgctccacgagacctggtgctgtctgagccaagcagccaatccttgagagtacagtggacagcggccagtggccctgtgactggctacaaggtccagtacactcctctgacggggctgggacagccactgccgagtgagcggcaggaggtgaacgtcccagctggtgagaccagtgtgcggctgcggggtctccggccactgaccgagtaccaagtgactgtgattgccctctacgccaacagcatcggggaggctgtgagcgggacagctcggaccactgccctagaagggccggaactgaccatccagaataccacagcccacagcctcctggtggcctggcggagtgtgccaggtgccactggctaccgtgtgacatggcgggtcctcagtggtgggcccacacagcagcaggagctgggccctgggcagggttcagtgttgctgcgtgacttggagcctggcacggactatgaggtgaccgtgagcaccctatttggccgcagtgtggggcccgccacttccctgatggctcgcactgacgcttctgttgagcagaccctgcgcccggtcatcctgggccccacatccatcctcctttcctggaacttggtgcctgaggcccgtggctaccggttggaatggcggcgtgagactggcttggagccaccgcagaaggtggtactgccctctgatgtgacccgctaccagttggatgggctgcagccgggcactgagtaccgcctcacactctacactctgctggagggccacgaggtggccacccctgcaaccgtggttcccactggaccagagctgcctgtgagccctgtaacagacctgcaagccaccgagctgcccgggcagcgggtgcgagtgtcctggagcccagtccctggtgccacccagtaccgcatcattgtgcgcagcacccagggggttgagcggaccctggtgcttcctgggagtcagacagcattcgacttggatgacgttcaggctgggcttagctacactgtgcgggtgtctgctcgagtgggtccccgtgagggcagtgccagtgtcctcactgtccgccgggagccggaaactccacttgctgttccagggctgcgggttgtggtgtcagatgcaacgcgagtgagggtggcctggggacccgtccctggagccagtggatttcggattagctggagcacaggcagtggtccggagtccagccagacactgcccccagactctactgccacagacatcacagggctgcagcctggaaccacctaccaggtggctgtgtcggtactgcgaggcagagaggagggccctgctgcagtcatcgtggctcgaacggacccactgggcccagtgaggacggtccatgtgactcaggccagcagctcatctgtcaccattacctggaccagggttcctggcgccacaggatacagggtttcctggcactcagcccacggcccagagaaatcccagttggtttctggggaggccacggtggctgagctggatggactggagccagatactgagtatacggtgcatgtgagggcccatgtggctggcgtggatgggccccctgcctctgtggttgtgaggactgcccctgagcctgtgggtcgtgtgtcgaggctgcagatcctcaatgcttccagcgacgttctacggatcacctgggtaggggtcactggagccacagcttacagactggcctggggccggagtgaaggcggccccatgaggcaccagatactcccaggaaacacagactctgcagagatccggggtctcgaaggtggagtcagctactcagtgcgagtgactgcacttgtcggggaccgcgagggcacacctgtctccattgttgtcactacgccgcctgaggctccgccagccctggggacgcttcacgtggtgcagcgcggggagcactcgctgaggctgcgctgggagccggtgcccagagcgcagggcttccttctgcactggcaacctgagggtggccaggaacagtcccgggtcctggggcccgagctcagcagctatcacctggacgggctggagccagcgacacagtaccgcgtgaggctgagtgtcctagggccagctggagaagggccctctgcagaggtgactgcgcgcactgagtcacctcgtgttccaagcattgaactacgtgtggtggacacctcgatcgactcggtgactttggcctggactccagtgtccagggcatccagctacatcctatcctggcggccactcagaggccctggccaggaagtgcctgggtccccgcagacacttccagggatctcaagctcccagcgggtgacagggctagagcctggcgtctcttacatcttctccctgacgcctgtcctggatggtgtgcggggtcctgaggcatctgtcacacagacgccagtgtgcccccgtggcctggcggatgtggtgttcctaccacatgccactcaagacaatgctcaccgtgcggaggctacgaggagggtcctggagcgtctggtgttggcacttgggcctcttgggccacaggcagttcaggttggcctgctgtcttacagtcatcggccctccccactgttcccactgaatggctcccatgaccttggcattatcttgcaaaggatccgtgacatgccctacatggacccaagtgggaacaacctgggcacagccgtggtcacagctcacagatacatgttggcaccagatgctcctgggcgccgccagcacgtaccaggggtgatggttctgctagtggatgaacccttgagaggtgacatattcagccccatccgtgaggcccaggcttctgggcttaatgtggtgatgttgggaatggctggagcggacccagagcagctgcgtcgcttggcgccgggtatggactctgtccagaccttcttcgccgtggatgatgggccaagcctggaccaggcagtcagtggtctggccacagccctgtgtcaggcatccttcactactcagccccggccagagccctgcccagtgtattgtccaaagggccagaagggggaacctggagagatgggcctgagaggacaagttgggcctcctggcgaccctggcctcccgggcaggaccggtgctcccggcccccaggggccccctggaagtgccactgccaagggcgagaggggcttccctggagcagatgggcgtccaggcagccctggccgcgccgggaatcctgggacccctggagcccctggcctaaagggctctccagggttgcctggccctcgtggggacccgggagagcgaggacctcgaggcccaaagggggagccgggggctcccggacaagtcatcggaggtgaaggacctgggcttcctgggcggaaaggggaccctggaccatcgggcccccctggacctcgtggaccactgggggacccaggaccccgtggccccccagggcttcctggaacagccatgaagggtgacaaaggcgatcgtggggagcggggtccccctggaccaggtgaaggtggcattgctcctggggagcctgggctgccgggtcttcccggaagccctggaccccaaggccccgttggcccccctggaaagaaaggagaaaaaggtgactctgaggatggagctccaggcctcccaggacaacctgggtctccgggtgagcagggcccacggggacctcctggagctattggccccaaaggtgaccggggctttccagggcccctgggtgaggctggagagaagggcgaacgtggacccccaggcccagcgggatcccgggggctgccaggggttgctggacgtcctggagccaagggtcctgaagggccaccaggacccactggccgccaaggagagaagggggagcctggtcgccctggggaccctgcagtggtgggacctgctgttgctggacccaaaggagaaaagggagatgtggggcccgctgggcccagaggagctaccggagtccaaggggaacggggcccacccggcttggttcttcctggagaccctggccccaagggagaccctggagaccggggtcccattggccttactggcagagcaggacccccaggtgactcagggcctcctggagagaagggagaccctgggcggcctggccccccaggacctgttggcccccgaggacgagatggtgaagttggagagaaaggtgacgagggtcctccgggtgacccgggtttgcctggaaaagcaggcgagcgtggccttcggggggcacctggagttcgggggcctgtgggtgaaaagggagaccagggagatcctggagaggatggacgaaatggcagccctggatcatctggacccaagggtgaccgtggggagccgggtcccccaggacccccgggacggctggtagacacaggacctggagccagagagaagggagagcctggggaccgcggacaagagggtcctcgagggcccaagggtgatcctggcctccctggagcccctggggaaaggggcattgaagggtttcggggacccccaggcccacagggggacccaggtgtccgaggcccagcaggagaaaagggtgaccggggtccccctgggctggatggccggagcggactggatgggaaaccaggagccgctgggccctctgggccgaatggtgctgcaggcaaagctggggacccagggagagacgggcttccaggcctccgtggagaacagggcctccctggcccctctggtccccctggattaccgggaaagccaggcgaggatggcaaacctggcctgaatggaaaaaacggagaacctggggaccctggagaagacgggaggaagggagagaaaggagattcaggcgcctctgggagagaaggtcgtgatggccccaagggtgagcgtggagctcctggtatccttggaccccaggggcctccaggcctcccagggccagtgggccctcctggccagggttttcctggtgtcccaggaggcacgggccccaagggtgaccgtggggagactggatccaaaggggagcagggcctccctggagagcgtggcctgcgaggagagcctggaagtgtgccgaatgtggatcggttgctggaaactgctggcatcaaggcatctgccctgcgggagatcgtggagacctgggatgagagctctggtagcttcctgcctgtgcccgaacggcgtcgaggccccaagggggactcaggcgaacagggccccccaggcaaggagggccccatcggctttcctggagaacgcgggctgaagggcgaccgtggagaccctggccctcaggggccacctggtctggcccttggggagaggggcccccccgggccttccggccttgccggggagcctggaaagcctggtattcccgggctcccaggcagggctgggggtgtgggagaggcaggaaggccaggagagaggggagaacggggagagaaaggagaacgtggagaacagggcagagatggccctcctggactccctggaacccctgggccccccggaccccctggccccaaggtgtctgtggatgagccaggtcctggactctctggagaacagggaccccctggactcaagggtgctaagggggagccgggcagcaatggtgaccaaggtcccaaaggagacaggggtgtgccaggcatcaaaggagaccggggagagcctggaccgaggggtcaggacggcaacccgggtctaccaggagagcgtggtatggctgggcctgaagggaagccgggtctgcagggtccaagaggcccccctggcccagtgggtggtcatggagaccctggaccacctggtgccccgggtcttgctggccctgcaggaccccaaggaccttctggcctgaagggggagcctggagagacaggacctccaggacggggcctgactggacctactggagctgtgggacttcctggaccccccggcccttcaggccttgtgggtccacaggggtctccaggtttgcctggacaagtgggggagacagggaagccgggagccccaggtcgagatggtgccagtggaaaagatggagacagagggagccctggtgtgccagggtcaccaggtctgcctggccctgtcggacctaaaggagaacctggccccacgggggcccctggacaggctgtggtcgggctccctggagcaaagggagagaagggagcccctggaggccttgctggagacctggtgggtgagccgggagccaaaggtgaccgaggactgccagggccgcgaggcgagaagggtgaagctggccgtgcaggggagcccggagaccctggggaagatggtcagaaaggggctccaggacccaaaggtttcaagggtgacccaggagtcggggtcccgggctcccctgggcctcctggccctccaggtgtgaagggagatctgggcctccctggcctgcccggtgctcctggtgttgttgggttcccgggtcagacaggccctcgaggagagatgggtcagccaggccctagtggagagcggggtctggcaggccccccagggagagaaggaatcccaggacccctggggccacctggaccaccggggtcagtgggaccacctggggcctctggactcaaaggagacaagggagaccctggagtagggctgcctgggccccgaggcgagcgtggggagccaggcatccggggtgaagatggccgccccggccaggagggaccccgaggactcacggggccccctggcagcaggggagagcgtggggagaagggtgatgttgggagtgcaggactaaagggtgacaagggagactcagctgtgatcctggggcctccaggcccacggggtgccaagggggacatgggtgaacgagggcctcggggcttggatggtgacaaaggacctcggggagacaatggggaccctggtgacaagggcagcaagggagagcctggtgacaagggctcagccgggttgccaggactgcgtggactcctgggaccccagggtcaacctggtgcagcagggatccctggtgacccgggatccccaggaaaggatggagtgcctggtatccgaggagaaaaaggagatgttggcttcatgggtccccggggcctcaagggtgaacggggagtgaagggagcctgtggccttgatggagagaagggagacaagggagaagctggtcccccaggccgccccgggctggcaggacacaaaggagagatgggggagcctggtgtgccgggccagtcgggggcccctggcaaggagggcctgatcggtcccaagggtgaccgaggctttgacgggcagccaggccccaagggtgaccagggcgagaaaggggagcggggaaccccaggaattgggggcttcccaggccccagtggaaatgatggctctgctggtcccccagggccacctggcagtgttggtcccagaggccccgaaggacttcagggccagaagggtgagcgaggtccccccggagagagagtggtgggggctcctggggtccctggagctcctggcgagagaggggagcaggggcggccagggcctgccggtcctcgaggcgagaagggagaagctgcactgacggaggatgacatccggggctttgtgcgccaagagatgagtcagcactgtgcctgccagggccagttcatcgcatctggatcacgacccctccctagttatgctgcagacactgccggctcccagctccatgctgtgcctgtgctccgcgtctctcatgcagaggaggaagagcgggtaccccctgaggatgatgagtactctgaatactccgagtattctgtggaggagtaccaggaccctgaagctccttgggatagtgatgacccctgttccctgccactggatgagggctcctgcactgcctacaccctgcgctggtaccatcgggctgtgacaggcagcacagaggcctgtcacccttttgtctatggtggctgtggagggaatgccaaccgttttgggacccgtgaggcctgcgagcgccgctgcccaccccgggtggtccagagccaggggacaggtactgcccaggactgaggcccagataatgagctgagattcagcatcccctggaggagtcggggtctcagcagaaccccactgtccctccccttggtgctagaggcttgtgtgcacgtgagcgtgcgtgtgcacgtccgttatttcagtgacttggtcccgtgggtctagccttcccccctgtggacaaacccccattgtggctcctgccaccctggcagatgactcactgtgggggggtggctgtgggcagtgagcggatgtgactggcgtctgacccgccccttgacccaagcctgtgatgacatggtgctgattctggggggcattaaagctgctgttttaaaaggc

SEQ ID NO: 2 - protein, 2944 aa, Homo sapiens
MTLRLLVAALCAGILAEAPRVRAQHRERVTCTRLYAADIVFLLDGSSSIGRSNFREVRSFLEGLVLPFSGAASAQGVRFATVQYSDDPRTEFGLDALGSGGDVIRAIRELSYKGGNTRTGAAILHVADHVFLPQLARPGVPKVCILITDGKSQDLVDTAAQRLKGQGVKLFAVGIKNADPEELKRVASQPTSDFFFFVNDFSILRTLLPLVSRRVCTTAGGVPVTRPPDDSTSAPRDLVLSEPSSQSLRVQWTAASGPVTGYKVQYTPLTGLGQPLPSERQEVNVPAGETSVRLRGLRPLTEYQVTVIALYANSIGEAVSGTARTTALEGPELTIQNTTAHSLLVAWRSVPGATGYRVTWRVLSGGPTQQQELGPGQGSVLLRDLEPGTDYEVTVSTLFGRSVGPATSLMARTDASVEQTLRPVILGPTSILLSWNLVPEARGYRLEWRRETGLEPPQKVVLPSDVTRYQLDGLQPGTEYRLTLYTLLEGHEVATPATVVPTGPELPVSPVTDLQATELPGQRVRVSWSPVPGATQYRIIVRSTQGVERTLVLPGSQTAFDLDDVQAGLSYTVRVSARVGPREGSASVLTVRREPETPLAVPGLRVVVSDATRVRVAWGPVPGASGFRISWSTGSGPESSQTLPPDSTATDITGLQPGTTYQVAVSVLRGREEGPAAVIVARTDPLGPVRTVHVTQASSSSVTITWTRVPGATGYRVSWHSAHGPEKSQLVSGEATVAELDGLEPDTEYTVHVRAHVAGVDGPPASVVVRTAPEPVGRVSRLQILNASSDVLRITWVGVTGATAYRLAWGRSEGGPMRHQILPGNTDSAEIRGLEGGVSYSVRVTALVGDREGTPVSIVVTTPPEAPPALGTLHVVQRGEHSLRLRWEPVPRAQGFLLHWQPEGGQEQSRVLGPELSSYHLDGLEPATQYRVRLSVLGPAGEGPSAEVTARTESPRVPSIELRVVDTSIDSVTLAWTPVSRASSYILSWRPLRGPGQEVPGSPQTLPGISSSQRVTGLEPGVSYIFSLTPVLDGVRGPEASVTQTPVCPRGLADVVFLPHATQDNAHRAEATRRVLERLVLALGPLGPQAVQVGLLSYSHRPSPLFPLNGSHDLGIILQRIRDMPYMDPSGNNLGTAVVTAHRYMLAPDAPGRRQHVPGVMVLLVDEPLRGDIFSPIREAQASGLNVVMLGMAGADPEQLRRLAPGMDSVQTFFAVDDGPSLDQAVSGLATALCQASFTTQPRPEPCPVYCPKGQKGEPGEMGLRGQVGPPGDPGLPGRTGAPGPQGPPGSATAKGERGFPGADGRPGSPGRAGNPGTPGAPGLKGSPGLPGPRGDPGERGPRGPKGEPGAPGQVIGGEGPGLPGRKGDPGPSGPPGPRGPLGDPGPRGPPGLPGTAMKGDKGDRGERGPPGPGEGGIAPGEPGLPGLPGSPGPQGPVGPPGKKGEKGDSEDGAPGLPGQPGSPGEQGPRGPPGAIGPKGDRGFPGPLGEAGEKGERGPPGPAGSRGLPGVAGRPGAKGPEGPPGPTGRQGEKGEPGRPGDPAVVGPAVAGPKGEKGDVGPAGPRGATGVQGERGPPGLVLPGDPGPKGDPGDRGPIGLTGRAGPPGDSGPPGEKGDPGRPGPPGPVGPRGRDGEVGEKGDEGPPGDPGLPGKAGERGLRGAPGVRGPVGEKGDQGDPGEDGRNGSPGSSGPKGDRGEPGPPGPPGRLVDTGPGAREKGEPGDRGQEGPRGPKGDPGLPGAPGERGIEGFRGPPGPQGDPGVRGPAGEKGDRGPPGLDGRSGLDGKPGAAGPSGPNGAAGKAGDPGRDGLPGLRGEQGLPGPSGPPGLPGKPGEDGKPGLNGKNGEPGDPGEDGRKGEKGDSGASGREGRDGPKGERGAPGILGPQGPPGLPGPVGPPGQGFPGVPGGTGPKGDRGETGSKGEQGLPGERGLRGEPGSVPNVDRLLETAGIKASALREIVETWDESSGSFLPVPERRRGPKGDSGEQGPPGKEGPIGFPGERGLKGDRGDPGPQGPPGLALGERGPPGPSGLAGEPGKPGIPGLPGRAGGVGEAGRPGERGERGEKGERGEQGRDGPPGLPGTPGPPGPPGPKVSVDEPGPGLSGEQGPPGLKGAKGEPGSNGDQGPKGDRGVPGIKGDRGEPGPRGQDGNPGLPGERGMAGPEGKPGLQGPRGPPGPVGGHGDPGPPGAPGLAGPAGPQGPSGLKGEPGETGPPGRGLTGPTGAVGLPGPPGPSGLVGPQGSPGLPGQVGETGKPGAPGRDGASGKDGDRGSPGVPGSPGLPGPVGPKGEPGPTGAPGQAVVGLPGAKGEKGAPGGLAGDLVGEPGAKGDRGLPGPRGEKGEAGRAGEPGDPGEDGQKGAPGPKGFKGDPGVGVPGSPGPPGPPGVKGDLGLPGLPGAPGVVGFPGQTGPRGEMGQPGPSGERGLAGPPGREGIPGPLGPPGPPGSVGPPGASGLKGDKGDPGVGLPGPRGERGEPGIRGEDGRPGQEGPRGLTGPPGSRGERGEKGDVGSAGLKGDKGDSAVILGPPGPRGAKGDMGERGPRGLDGDKGPRGDNGDPGDKGSKGEPGDKGSAGLPGLRGLLGPQGQPGAAGIPGDPGSPGKDGVPGIRGEKGDVGFMGPRGLKGERGVKGACGLDGEKGDKGEAGPPGRPGLAGHKGEMGEPGVPGQSGAPGKEGLIGPKGDRGFDGQPGPKGDQGEKGERGTPGIGGFPGPSGNDGSAGPPGPPGSVGPRGPEGLQGQKGERGPPGERVVGAPGVPGAPGERGEQGRPGPAGPRGEKGEAALTEDDIRGFVRQEMSQHCACQGQFIASGSRPLPSYAADTAGSQLHAVPVLRVSHAEEEERVPPEDDEYSEYSEYSVEEYQDPEAPWDSDDPCSLPLDEGSCTAYTLRWYHRAVTGSTEACHPFVYGGCGGNANRFGTREACERRCPPRVVQSQGTGTAQD

SEQ ID NO: 3 - DNA, 53 bp, Artificial Sequence
  Description of Artificial Sequence: Synthetic primer
cgacttgtgttgggactggctagcgccaccatgacgctgcggcttctggtggc

SEQ ID NO: 4 - DNA, 22 bp, Artificial Sequence
  Description of Artificial Sequence: Synthetic primer
gggcttagctacactgtgcggg

SEQ ID NO: 5 - DNA, 24 bp, Artificial Sequence
  Description of Artificial Sequence: Synthetic primer
cctgcccagtgtattgtccaaagg

SEQ ID NO: 6 - DNA, 21 bp, Artificial Sequence
  Description of Artificial Sequence: Synthetic primer
ctgctggcatcaaggcatctg

SEQ ID NO: 7 - DNA, 22 bp, Artificial Sequence
  Description of Artificial Sequence: Synthetic primer
cccgcacagtgtagctaagccc

SEQ ID NO: 8 - DNA, 24 bp, Artificial Sequence
  Description of Artificial Sequence: Synthetic primer
cctttggacaatacactgggcagg

SEQ ID NO: 9 - DNA, 21 bp, Artificial Sequence
  Description of Artificial Sequence: Synthetic primer
cagatgccttgatgccagcag

SEQ ID NO: 10 - DNA, 53 bp, Artificial Sequence
  Description of Artificial Sequence: Synthetic primer
cgtgatttcatttgctacacgtaatcgattcagtcctgggcagtacctgtccc

SEQ ID NO: 11 - DNA, 341 bp, Artificial Sequence
  Description of Artificial Sequence: Synthetic polynucleotide
cgctcccagaacatcacctaccactgcaagaacagcgtggcctacatggaccagcagactggcaacctcaagaaggccctgctcctccagggctccaacgagatcgagatccgcgccgagggcaacagccgcttcacctacagcgtcactgtcgatggctgcacgagtcacaccggagcctggggcaagacagtgattgaatacaaaaccaccaagacctcccgcctgcgcatcatcgatgtggcccccttggacgttggtgccccagaccaggaattcggcttcgacgttggccatgtctgcttcctgtaaatcgattacgtgtagcaaatgaaatcacg

SEQ ID NO: 12 - DNA, 730 bp, Artificial Sequence
  Description of Artificial Sequence: Synthetic polynucleotide
ttcaaattttcgggggatcgcattagttattaatagtaatcaattacggggtcattagttcatagcccatatatggagttccgcgttacataacttacggtaaatggcccgcctggttgaccgcccaacgacccccgcccattgacgtcaataatgacgtatgttcccatagtaacgccaatagggactttccattgacgtcaatgggtggagtatttacggtaaactgcccacttggtagtacatcaagtgtatcatacgccaagtacgccccctattgacgtcaatgacggtaaatggcccgcctggtattatgcccagtacatgaccttatgggactttcctacttggcagtacatctgcgtattagtcatcgctattaccatggtgatgcggttttggcagtacatcaatgggcgtggatagcggtttgactcacggggatttccaagtctccaccccattgacgtcaatgggagtttgttttggcaccaaaatcaacgggactttccaaaatgtcgtaacaactccgccccattgacgcaaatgggcggtaggcgtgtacggtgggaggtctatataagcagagctggtttagtgaaccgtcagatccgctagcattgtgtgcttttcgggccaccatgacgctgcggcttctggtggccgcgctctgcgccgggatcctggcagaggcgccccgagtgcgagcccagcacagggagagagtgac

SEQ ID NO: 13 - DNA, 740 bp, Artificial Sequence
  Description of Artificial Sequence: Synthetic polynucleotide
agtgcgagcccagcacagggagagagtgacctgcacgcgcctttacgccgctgacattgtgttcttactggatggctcctcatccattggccgcagcaatttccgcgaggtccgcagctttctcgaagggctggtgctgcctttctctggagcagccagtgcacagggtgtgcgctttgccacagtgcagtacagcgatgacccacggacagagttcggcctggatgcacttggctctgggggtgatgtgatccgcgccatccgtgagcttagctacaaggggggcaacactcgcacaggggctgcaattctccatgtggctgaccatgtcttcctgccccagctggcccgacctggtgtccccaaggtctgcatcctgatcacgtctctcatgcagaggaggaagagcgggtaccccctgaggatgatgagtactctgaatactccgagtattctgtggaggagtaccaggaccctgaagctccttgggatagtgatgacccctgttccctgccactggatgagggctcctgcactgcctacaccctgcgctggtaccatcgggctgtgacaggcagcacagaggcctgtcacccttttgtctatggtggctgtggagggaatgccaaccgttttgggacccgtgaggcctgcgagcgccgctgcccaccccgggtggtccagagccaggggacaggtactgcccaggactgagtacctttaagaccaatgacttacaa

SEQ ID NO: 14 - DNA, 20 bp, Artificial Sequence
  Description of Artificial Sequence: Synthetic primer
atggaaaaacgccagcaacg

SEQ ID NO: 15 - DNA, 20 bp, Artificial Sequence
  Description of Artificial Sequence: Synthetic primer
ctgtcacccttttgtctatg

SEQ ID NO: 16 - DNA, 24 bp, Artificial Sequence
  Description of Artificial Sequence: Synthetic primer
gttgccggacacttcttgtcctct

SEQ ID NO: 17 - DNA, 22 bp, Artificial Sequence
  Description of Artificial Sequence: Synthetic primer
cccgcacagtgtagctaagccc

SEQ ID NO: 18 - DNA, 20 bp, Artificial Sequence
  Description of Artificial Sequence: Synthetic primer
agaggccccgaaggacttca

SEQ ID NO: 19 - DNA, 467 bp, Artificial Sequence
  Description of Artificial Sequence: Synthetic polynucleotide
acagcagagatccagtttggttaattaagcattagttattaatagtaatcaattacggggtcattaagactcggccttagaaccccagtatcagcagaaccgcgtctctcatgcagaggaggaagagcgggtaccccctgaggatgatgagtactctgaatactccgagtattctgtggaggagtaccaggaccctgaagctccttgggatagtgatgacccctgttccctgccactggatgagggctcctgcactgcctacaccctgcgctggtaccatcgggctgtgacaggcagcacagaggcctgtcacccttttgtctatggtggctgtggagggaatgccaaccgttttgggacccgtgaggcctgcgagcgccgctgcccaccccgggtggtccagagccaggggacaggtactgcccaggactgatcgataccgtcgacctcgagacctagaaaaacat

SEQ ID NO: 20 - DNA, 21 bp, Artificial Sequence
  Description of Artificial Sequence: Synthetic primer
gtagacataatagcaacagac

SEQ ID NO: 21 - DNA, 21 bp, Artificial Sequence
  Description of Artificial Sequence: Synthetic primer
tattgctacttgtgattgctc

SEQ ID NO: 22 - DNA, 20 bp, Artificial Sequence
  Description of Artificial Sequence: Synthetic primer
agaggccccgaaggacttca

SEQ ID NO: 23 - DNA, 8832 bp, Artificial Sequence
  Description of Artificial Sequence: Synthetic polynucleotide
atgacgctgcggcttctggtggccgcgctctgcgccgggatcctggcagaggcgccccgagtgcgagcccagcacagggagagagtgacctgcacgcgcctttacgccgctgacattgtgttcttactggatggctcctcatccattggccgcagcaatttccgcgaggtccgcagctttctcgaagggctggtgctgcctttctctggagcagccagtgcacagggtgtgcgctttgccacagtgcagtacagcgatgacccacggacagagttcggcctggatgcacttggctctgggggtgatgtgatccgcgccatccgtgagcttagctacaaggggggcaacactcgcacaggggctgcaattctccatgtggctgaccatgtcttcctgccccagctggcccgacctggtgtccccaaggtctgcatcctgatcacagacgggaagtcccaggacctggtggacacagctgcccaaaggctgaaggggcagggggtcaagctatttgctgtggggatcaagaatgctgaccctgaggagctgaagcgagttgcctcacagcccaccagtgacttcttcttcttcgtcaatgacttcagcatcttgaggacactactgcccctcgtttcccggagagtgtgcacgactgctggtggcgtgcctgtgacccgacctccggatgactcgacctctgctccacgagacctggtgctgtctgagccaagcagccaatccttgagagtacagtggacagcggccagtggccctgtgactggctacaaggtccagtacactcctctgacggggctgggacagccactgccgagtgagcggcaggaggtgaacgtcccagctggtgagaccagtgtgcggctgcggggtctccggccactgaccgagtaccaagtgactgtgattgccctctacgccaacagcatcggggaggctgtgagcgggacagctcggaccactgccctagaagggccggaactgaccatccagaataccacagcccacagcctcctggtggcctggcggagtgtgccaggtgccactggctaccgtgtgacatggcgggtcctcagtggtgggcccacacagcagcaggagctgggccctgggcagggttcagtgttgctgcgtgacttggagcctggcacggactatgaggtgaccgtgagcaccctatttggccgcagtgtggggcccgccacttccctgatggctcgcactgacgcttctgttgagcagaccctgcgcccggtcatcctgggccccacatccatcctcctttcctggaacttggtgcctgaggcccgtggctaccggttggaatggcggcgtgagactggcttggagccaccgcagaaggtggtactgccctctgatgtgacccgctaccagttggatgggctgcagccgggcactgagtaccgcctcacactctacactctgctggagggccacgaggtggccacccctgcaaccgtggttcccactggaccagagctgcctgtgagccctgtaacagacctgcaagccaccgagctgcccgggcagcgggtgcgagtgtcctggagcccagtccctggtgccacccagtaccgcatcattgtgcgcagcacccagggggttgagcggaccctggtgcttcctgggagtcagacagcattcgacttggatgacgttcaggctgggcttagctacactgtgcgggtgtctgctcgagtgggtccccgtgagggcagtgccagtgtcctcactgtccgccgggagccggaaactccacttgctgttccagggctgcgggttgtggtgtcagatgcaacgcgagtgagggtggcctggggacccgtccctggagccagtggatttcggattagctggagcacaggcagtggtccggagtccagccagacactgcccccagactctactgccacagacatcacagggctgcagcctggaaccacctaccaggtggctgtgtcggtactgcgaggcagagaggagggccctgctgcagtcatcgtggctcgaacggacccactgggcccagtgaggacggtccatgtgactcaggccagcagctcatctgtcaccattacctggaccagggttcctggcgccacaggatacagggtttcctggcactcagcccacggcccagagaaatcccagttggtttctggggaggccacggtggctgagctggatggactggagccagatactgagtatacggtgcatgtgagggcccatgtggctggcgtggatgggccccctgcctctgtggttgtgaggactgcccctgagcctgtgggtcgtgtgtcgaggctgcagatcctcaatgcttccagcgacgttctacggatcacctgggtaggggtcactggagccacagcttacagactggcctggggccggagtgaaggcggccccatgaggcaccagatactcccaggaaacacagactctgcagagatccggggtctcgaaggtggagtcagctactcagtgcgagtgactgcacttgtcggggaccgcgagggcacacctgtctccattgttgtcactacgccgcctgaggctccgccagccctggggacgcttcacgtggtgcagcgcggggagcactcgctgaggctgcgctgggagccggtgcccagagcgcagggcttccttctgcactggcaacctgagggtggccaggaacagtcccgggtcctggggcccgagctcagcagctatcacctggacgggctggagccagcgacacagtaccgcgtgaggctgagtgtcctagggccggctggagaagggccctctgcagaggtgactgcgcgcactgagtcacctcgtgttccaagcattgaactacgtgtggtggacacctcgatcgactcggtgactttggcctggactccagtgtccagggcatccagctacatcctatcctggcggccactcagaggccctggccaggaagtgcctgggtccccgcagacacttccagggatctcaagctcccagcgggtgacagggctagagcctggcgtctcttacatcttctccctgacgcctgtcctggatggtgtgcggggtcctgaggcatctgtcacacagacgccagtgtgcccccgtggcctggcggatgtggtgttcctaccacatgccactcaagacaatgctcaccgtgcggaggctacgaggagggtcctggagcgtctggtgttggcacttgggcctcttgggccacaggcagttcaggttggcctgctgtcttacagtcatcggccctccccactgttcccactgaatggctcccatgaccttggcattatcttgcaaaggatccgtgacatgccctacatggacccaagtgggaacaacctgggcacagccgtggtcacagctcacagatacatgttggcaccagatgctcctgggcgccgccagcacgtaccaggggtgatggttctgctagtggatgaacccttgagaggtgacatattcagccccatccgtgaggcccaggcttctgggcttaatgtggtgatgttgggaatggctggagcggacccagagcagctgcgtcgcttggcgccgggtatggactctgtccagaccttcttcgccgtggatgatgggccaagcctggaccaggcagtcagtggtctggccacagccctgtgtcaggcatccttcactactcagccccggccagagccctgcccagtgtattgtccaaagggccagaagggggaacctggagagatgggcctgagaggacaagttgggcctcctggcgaccctggcctcccgggcaggaccggtgctcccggcccccaggggccccctggaagtgccactgccaagggcgagaggggcttccctggagcagatgggcgtccaggcagccctggccgcgccgggaatcctgggacccctggagcccctggcctaaagggctctccagggttgcctggccctcgtggggacccgggagagcgaggacctcgaggcccaaagggggagccgggggctcccggacaagtcatcggaggtgaaggacctgggcttcctgggcggaaaggggaccctggaccatcgggcccccctggacctcgtggaccactgggggacccaggaccccgtggccccccagggcttcctggaacagccatgaagggtgacaaaggcgatcgtggggagcggggtccccctggaccaggtgaaggtggcattgctcctggggagcctgggctgccgggtcttcccggaagccctggaccccaaggccccgttggcccccctggaaagaaaggagaaaaaggtgactctgaggatggagctccaggcctcccaggacaacctgggtctccgggtgagcagggcccacggggacctcctggagctattggccccaaaggtgaccggggctttccagggcccctgggtgaggctggagagaagggcgaacgtggacccccaggcccagcgggatcccgggggctgccaggggttgctggacgtcctggagccaagggtcctgaagggccaccaggacccactggccgccaaggagagaagggggagcctggtcgccctggggaccctgcagtggtgggacctgctgttgctggacccaaaggagaaaagggagatgtggggcccgctgggcccagaggagctaccggagtccaaggggaacggggcccacccggcttggttcttcctggagaccctggccccaagggagaccctggagaccggggtcccattggccttactggcagagcaggacccccaggtgactcagggcctcctggagagaagggagaccctgggcggcctggccccccaggacctgttggcccccgaggacgagatggtgaagttggagagaaaggtgacgagggtcctccgggtgacccgggtttgcctggaaaagcaggcgagcgtggccttcggggggcacctggagttcgggggcctgtgggtgaaaagggagaccagggagatcctggagaggatggacgaaatggcagccctggatcatctggacccaagggtgaccgtggggagccgggtcccccaggacccccgggacggctggtagacacaggacctggagccagagagaagggagagcctggggaccgcggacaagagggtcctcgagggcccaagggtgatcctggcctccctggagcccctggggaaaggggcattgaagggtttcggggacccccaggcccacagggggacccaggtgtccgaggcccagcaggagaaaagggtgaccggggtccccctgggctggatggccggagcggactggatgggaaaccaggagccgctgggccctctgggccgaatggtgctgcaggcaaagctggggacccagggagagacgggcttccaggcctccgtggagaacaaggcctccctggcccctctggtccccctggattaccgggaaagccaggcgaggatgggaaacctggcctgaatggaaaaaacggagaacctggggaccctggagaagacgggaggaagggagagaaaggagattcaggcgcctctgggagagaaggtcgtgatggccccaagggtgagcgtggagctcctggtatccttggaccccaggggcctccaggcctcccagggccagtgggccctcctggccagggttttcctggtgtcccaggaggcacgggccccaagggtgaccgtggggagactggatccaaaggggagcagggcctccctggagagcgtggcctgcgaggagagcctggaagtgtgccgaatgtggatcggttgctggaaactgctggcatcaaggcatctgccctgcgggagatcgtggagacctgggatgagagctctggtagcttcctgcctgtgcccgaacggcgtcgaggccccaagggggactcaggcgaacagggccccccaggcaaggagggccccatcggctttcctggagaacgcgggctgaagggcgaccgtggagaccctggccctcaggggccacctggtctggcccttggggagaggggcccccccgggccttccggccttgccggggagcctggaaagcctggtattcccgggctcccaggcagggctgggggtgtgggagaggcaggaaggccaggagagaggggagaacggggagagaaaggagaacgtggagaacagggcagagatggccctcctggactccctggaacccctgggccccccggaccccctggccccaaggtgtctgtggatgagccaggtcctggactctctggagaacagggaccccctggactcaagggtgctaagggggagccgggcagcaatggtgaccaaggtcccaaaggagacaggggtgtgccaggcatcaaaggagaccggggagagcctggaccgaggggtcaggacggcaacccgggtctaccaggagagcgtggtatggctgggcctgaagggaagccgggtctgcagggtccaagaggcccccctggcccagtgggtggtcatggagaccctggaccacctggtgccccgggtcttgctggccctgcaggaccccaaggaccttctggcctgaagggggagcctggagagacaggacctccaggacggggcctgactggacctactggagctgtgggacttcctggaccccccggcccttcaggccttgtgggtccacaggggtctccaggtttgcctggacaagtgggggagacagggaagccgggagccccaggtcgagatggtgccagtggaaaagatggagacagagggagccctggtgtgccagggtcaccaggtctgcctggccctgtcggacctaaaggagaacctggccccacgggggcccctggacaggctgtggtcgggctccctggagcaaagggagagaagggagcccctggaggccttgctggagacctggtgggtgagccgggagccaaaggtgaccgaggactgccagggccgcgaggcgagaagggtgaagctggccgtgcaggggagcccggagaccctggggaagatggtcagaaaggggctccaggacccaaaggtttcaagggtgacccaggagtcggggtcccgggctcccctgggcctcctggccctccaggtgtgaagggagatctgggcctccctggcctgcccggtgctcctggtgttgttgggttcccgggtcagacaggccctcgaggagagatgggtcagccaggccctagtggagagcggggtctggcaggccccccagggagagaaggaatcccaggacccctggggccacctggaccaccggggtcagtgggaccacctggggcctctggactcaaaggagacaagggagaccctggagtagggctgcctgggccccgaggcgagcgtggggagccaggcatccggggtgaagatggccgccccggccaggagggaccccgaggactcacggggccccctggcagcaggggagagcgtggggagaagggtgatgttgggagtgcaggactaaagggtgacaagggagactcagctgtgatcctggggcctccaggcccacggggtgccaagggggacatgggtgaacgagggcctcggggcttggatggtgacaaaggacctcggggagacaatggggaccctggtgacaagggcagcaagggagagcctggtgacaagggctcagccgggttgccaggactgcgtggactcctgggaccccagggtcaacctggtgcagcagggatccctggtgacccgggatccccaggaaaggatggagtgcctggtatccgaggagaaaaaggagatgttggcttcatgggtccccggggcctcaagggtgaacggggagtgaagggagcctgtggccttgatggagagaagggagacaagggagaagctggtcccccaggccgccccgggctggcaggacacaaaggagagatgggggagcctggtgtgccgggccagtcgggggcccctggcaaggagggcctgatcggtcccaagggtgaccgaggctttgacgggcagccaggccccaagggtgaccagggcgagaaaggggagcggggaaccccaggaattgggggcttcccaggccccagtggaaatgatggctctgctggtcccccagggccacctggcagtgttggtcccagaggccccgaaggacttcagggccagaagggtgagcgaggtccccccggagagagagtggtgggggctcctggggtccctggagctcctggcgagagaggggagcaggggcggccagggcctgccggtcctcgaggcgagaagggagaagctgcactgacggaggatgacatccggggctttgtgcgccaagagatgagtcagcactgtgcctgccagggccagttcatcgcatctggatcacgacccctccctagttatgctgcagacactgccggctcccagctccatgctgtgcctgtgctccgcgtctctcatgcagaggaggaagagcgggtaccccctgaggatgatgagtactctgaatactccgagtattctgtggaggagtaccaggaccctgaagctccttgggatagtgatgacccctgttccctgccactggatgagggctcctgcactgcctacaccctgcgctggtaccatcgggctgtgacaggcagcacagaggcctgtcacccttttgtctatggtggctgtggagggaatgccaaccgttttgggacccgtgaggcctgcgagcgccgctgcccaccccgggtggtccagagccaggggacaggtactgcccaggac

SEQ ID NO: 24 - DNA, 8832 bp, Homo sapiens
atgacgctgcggcttctggtggccgcgctctgcgccgggatcctggcagaggcgccccgagtgcgagcccagcacagggagagagtgacctgcacgcgcctttacgccgctgacattgtgttcttactggatggctcctcatccattggccgcagcaatttccgcgaggtccgcagctttctcgaagggctggtgctgcctttctctggagcagccagtgcacagggtgtgcgctttgccacagtgcagtacagcgatgacccacggacagagttcggcctggatgcacttggctctgggggtgatgtgatccgcgccatccgtgagcttagctacaaggggggcaacactcgcacaggggctgcaattctccatgtggctgaccatgtcttcctgccccagctggcccgacctggtgtccccaaggtctgcatcctgatcacagacgggaagtcccaggacctggtggacacagctgcccaaaggctgaaggggcagggggtcaagctatttgctgtggggatcaagaatgctgaccctgaggagctgaagcgagttgcctcacagcccaccagtgacttcttcttcttcgtcaatgacttcagcatcttgaggacactactgcccctcgtttcccggagagtgtgcacgactgctggtggcgtgcctgtgacccgacctccggatgactcgacctctgctccacgagacctggtgctgtctgagccaagcagccaatccttgagagtacagtggacagcggccagtggccctgtgactggctacaaggtccagtacactcctctgacggggctgggacagccactgccgagtgagcggcaggaggtgaacgtcccagctggtgagaccagtgtgcggctgcggggtctccggccactgaccgagtaccaagtgactgtgattgccctctacgccaacagcatcggggaggctgtgagcgggacagctcggaccactgccctagaagggccggaactgaccatccagaataccacagcccacagcctcctggtggcctggcggagtgtgccaggtgccactggctaccgtgtgacatggcgggtcctcagtggtgggcccacacagcagcaggagctgggccctgggcagggttcagtgttgctgcgtgacttggagcctggcacggactatgaggtgaccgtgagcaccctatttggccgcagtgtggggcccgccacttccctgatggctcgcactgacgcttctgttgagcagaccctgcgcccggtcatcctgggccccacatccatcctcctttcctggaacttggtgcctgaggcccgtggctaccggttggaatggcggcgtgagactggcttggagccaccgcagaaggtggtactgccctctgatgtgacccgctaccagttggatgggctgcagccgggcactgagtaccgcctcacactctacactctgctggagggccacgaggtggccacccctgcaaccgtggttcccactggaccagagctgcctgtgagccctgtaacagacctgcaagccaccgagctgcccgggcagcgggtgcgagtgtcctggagcccagtccctggtgccacccagtaccgcatcattgtgcgcagcacccagggggttgagcggaccctggtgcttcctgggagtcagacagcattcgacttggatgacgttcaggctgggcttagctacactgtgcgggtgtctgctcgagtgggtccccgtgagggcagtgccagtgtcctcactgtccgccgggagccggaaactccacttgctgttccagggctgcgggttgtggtgtcagatgcaacgcgagtgagggtggcctggggacccgtccctggagccagtggatttcggattagctggagcacaggcagtggtccggagtccagccagacactgcccccagactctactgccacagacatcacagggctgcagcctggaaccacctaccaggtggctgtgtcggtactgcgaggcagagaggagggccctgctgcagtcatcgtggctcgaacggacccactgggcccagtgaggacggtccatgtgactcaggccagcagctcatctgtcaccattacctggaccagggttcctggcgccacaggatacagggtttcctggcactcagcccacggcccagagaaatcccagttggtttctggggaggccacggtggctgagctggatggactggagccagatactgagtatacggtgcatgtgagggcccatgtggctggcgtggatgggccccctgcctctgtggttgtgaggactgcccctgagcctgtgggtcgtgtgtcgaggctgcagatcctcaatgcttccagcgacgttctacggatcacctgggtaggggtcactggagccacagcttacagactggcctggggccggagtgaaggcggccccatgaggcaccagatactcccaggaaacacagactctgcagagatccggggtctcgaaggtggagtcagctactcagtgcgagtgactgcacttgtcggggaccgcgagggcacacctgtctccattgttgtcactacgccgcctgaggctccgccagccctggggacgcttcacgtggtgcagcgcggggagcactcgctgaggctgcgctgggagccggtgcccagagcgcagggcttccttctgcactggcaacctgagggtggccaggaacagtcccgggtcctggggcccgagctcagcagctatcacctggacgggctggagccagcgacacagtaccgcgtgaggctgagtgtcctagggccagctggagaagggccctctgcagaggtgactgcgcgcactgagtcacctcgtgttccaagcattgaactacgtgtggtggacacctcgatcgactcggtgactttggcctggactccagtgtccagggcatccagctacatcctatcctggcggccactcagaggccctggccaggaagtgcctgggtccccgcagacacttccagggatctcaagctcccagcgggtgacagggctagagcctggcgtctcttacatcttctccctgacgcctgtcctggatggtgtgcggggtcctgaggcatctgtcacacagacgccagtgtgcccccgtggcctggcggatgtggtgttcctaccacatgccactcaagacaatgctcaccgtgcggaggctacgaggagggtcctggagcgtctggtgttggcacttgggcctcttgggccacaggcagttcaggttggcctgctgtcttacagtcatcggccctccccactgttcccactgaatggctcccatgaccttggcattatcttgcaaaggatccgtgacatgccctacatggacccaagtgggaacaacctgggcacagccgtggtcacagctcacagatacatgttggcaccagatgctcctgggcgccgccagcacgtaccaggggtgatggttctgctagtggatgaacccttgagaggtgacatattcagccccatccgtgaggcccaggcttctgggcttaatgtggtgatgttgggaatggctggagcggacccagagcagctgcgtcgcttggcgccgggtatggactctgtccagaccttcttcgccgtggatgatgggccaagcctggaccaggcagtcagtggtctggccacagccctgtgtcaggcatccttcactactcagccccggccagagccctgcccagtgtattgtccaaagggccagaagggggaacctggagagatgggcctgagaggacaagttgggcctcctggcgaccctggcctcccgggcaggaccggtgctcccggcccccaggggccccctggaagtgccactgccaagggcgagaggggcttccctggagcagatgggcgtccaggcagccctggccgcgccgggaatcctgggacccctggagcccctggcctaaagggctctccagggttgcctggccctcgtggggacccgggagagcgaggacctcgaggcccaaagggggagccgggggctcccggacaagtcatcggaggtgaaggacctgggcttcctgggcggaaaggggaccctggaccatcgggcccccctggacctcgtggaccactgggggacccaggaccccgtggccccccagggcttcctggaacagccatgaagggtgacaaaggcgatcgtggggagcggggtccccctggaccaggtgaaggtggcattgctcctggggagcctgggctgccgggtcttcccggaagccctggaccccaaggccccgttggcccccctggaaagaaaggagaaaaaggtgactctgaggatggagctccaggcctcccaggacaacctgggtctccgggtgagcagggcccacggggacctcctggagctattggccccaaaggtgaccggggctttccagggcccctgggtgaggctggagagaagggcgaacgtggacccccaggcccagcgggatcccgggggctgccaggggttgctggacgtcctggagccaagggtcctgaagggccaccaggacccactggccgccaaggagagaagggggagcctggtcgccctggggaccctgcagtggtgggacctgctgttgctggacccaaaggagaaaagggagatgtggggcccgctgggcccagaggagctaccggagtccaaggggaacggggcccacccggcttggttcttcctggagaccctggccccaagggagaccctggagaccggggtcccattggccttactggcagagcaggacccccaggtgactcagggcctcctggagagaagggagaccctgggcggcctggccccccaggacctgttggcccccgaggacgagatggtgaagttggagagaaaggtgacgagggtcctccgggtgacccgggtttgcctggaaaagcaggcgagcgtggccttcggggggcacctggagttcgggggcctgtgggtgaaaagggagaccagggagatcctggagaggatggacgaaatggcagccctggatcatctggacccaagggtgaccgtggggagccgggtcccccaggacccccgggacggctggtagacacaggacctggagccagagagaagggagagcctggggaccgcggacaagagggtcctcgagggcccaagggtgatcctggcctccctggagcccctggggaaaggggcattgaagggtttcggggacccccaggcccacagggggacccaggtgtccgaggcccagcaggagaaaagggtgaccggggtccccctgggctggatggccggagcggactggatgggaaaccaggagccgctgggccctctgggccgaatggtgctgcaggcaaagctggggacccagggagagacgggcttccaggcctccgtggagaacagggcctccctggcccctctggtccccctggattaccgggaaagccaggcgaggatggcaaacctggcctgaatggaaaaaacggagaacctggggaccctggagaagacgggaggaagggagagaaaggagattcaggcgcctctgggagagaaggtcgtgatggccccaagggtgagcgtggagctcctggtatccttggaccccaggggcctccaggcctcccagggccagtgggccctcctggccagggttttcctggtgtcccaggaggcacgggccccaagggtgaccgtggggagactggatccaaaggggagcagggcctccctggagagcgtggcctgcgaggagagcctggaagtgtgccgaatgtggatcggttgctggaaactgctggcatcaaggcatctgccctgcgggagatcgtggagacctgggatgagagctctggtagcttcctgcctgtgcccgaacggcgtcgaggccccaagggggactcaggcgaacagggccccccaggcaaggagggccccatcggctttcctggagaacgcgggctgaagggcgaccgtggagaccctggccctcaggggccacctggtctggcccttggggagaggggcccccccgggccttccggccttgccggggagcctggaaagcctggtattcccgggctcccaggcagggctgggggtgtgggagaggcaggaaggccaggagagaggggagaacggggagagaaaggagaacgtggagaacagggcagagatggccctcctggactccctggaacccctgggccccccggaccccctggccccaaggtgtctgtggatgagccaggtcctggactctctggagaacagggaccccctggactcaagggtgctaagggggagccgggcagcaatggtgaccaaggtcccaaaggagacaggggtgtgccaggcatcaaaggagaccggggagagcctggaccgaggggtcaggacggcaacccgggtctaccaggagagcgtggtatggctgggcctgaagggaagccgggtctgcagggtccaagaggcccccctggcccagtgggtggtcatggagaccctggaccacctggtgccccgggtcttgctggccctgcaggaccccaaggaccttctggcctgaagggggagcctggagagacaggacctccaggacggggcctgactggacctactggagctgtgggacttcctggaccccccggcccttcaggccttgtgggtccacaggggtctccaggtttgcctggacaagtgggggagacagggaagccgggagccccaggtcgagatggtgccagtggaaaagatggagacagagggagccctggtgtgccagggtcaccaggtctgcctggccctgtcggacctaaaggagaacctggccccacgggggcccctggacaggctgtggtcgggctccctggagcaaagggagagaagggagcccctggaggccttgctggagacctggtgggtgagccgggagccaaaggtgaccgaggactgccagggccgcgaggcgagaagggtgaagctggccgtgcaggggagcccggagaccctggggaagatggtcagaaaggggctccaggacccaaaggtttcaagggtgacccaggagtcggggtcccgggctcccctgggcctcctggccctccaggtgtgaagggagatctgggcctccctggcctgcccggtgctcctggtgttgttgggttcccgggtcagacaggccctcgaggagagatgggtcagccaggccctagtggagagcggggtctggcaggccccccagggagagaaggaatcccaggacccctggggccacctggaccaccggggtcagtgggaccacctggggcctctggactcaaaggagacaagggagaccctggagtagggctgcctgggccccgaggcgagcgtggggagccaggcatccggggtgaagatggccgccccggccaggagggaccccgaggactcacggggccccctggcagcaggggagagcgtggggagaagggtgatgttgggagtgcaggactaaagggtgacaagggagactcagctgtgatcctggggcctccaggcccacggggtgccaagggggacatgggtgaacgagggcctcggggcttggatggtgacaaaggacctcggggagacaatggggaccctggtgacaagggcagcaagggagagcctggtgacaagggctcagccgggttgccaggactgcgtggactcctgggaccccagggtcaacctggtgcagcagggatccctggtgacccgggatccccaggaaaggatggagtgcctggtatccgaggagaaaaaggagatgttggcttcatgggtccccggggcctcaagggtgaacggggagtgaagggagcctgtggccttgatggagagaagggagacaagggagaagctggtcccccaggccgccccgggctggcaggacacaaaggagagatgggggagcctggtgtgccgggccagtcgggggcccctggcaaggagggcctgatcggtcccaagggtgaccgaggctttgacgggcagccaggccccaagggtgaccagggcgagaaaggggagcggggaaccccaggaattgggggcttcccaggccccagtggaaatgatggctctgctggtcccccagggccacctggcagtgttggtcccagaggccccgaaggacttcagggccagaagggtgagcgaggtccccccggagagagagtggtgggggctcctggggtccctggagctcctggcgagagaggggagcaggggcggccagggcctgccggtcctcgaggcgagaagggagaagctgcactgacggaggatgacatccggggctttgtgcgccaagagatgagtcagcactgtgcctgccagggccagttcatcgcatctggatcacgacccctccctagttatgctgcagacactgccggctcccagctccatgctgtgcctgtgctccgcgtctctcatgcagaggaggaagagcgggtaccccctgaggatgatgagtactctgaatactccgagtattctgtggaggagtaccaggaccctgaagctccttgggatagtgatgacccctgttccctgccactggatgagggctcctgcactgcctacaccctgcgctggtaccatcgggctgtgacaggcagcacagaggcctgtcacccttttgtctatggtggctgtggagggaatgccaaccgttttgggacccgtgaggcctgcgagcgccgctgcccaccccgggtggtccagagccaggggacaggtactgcccaggac

SEQ ID NO: 25 - DNA, 21 bp, Artificial Sequence
  Description of Artificial Sequence: Synthetic primer
acctgaaagcgaaagggaaac

SEQ ID NO: 26 - DNA, 23 bp, Artificial Sequence
  Description of Artificial Sequence: Synthetic primer
cacccatctctctccttctagcc

SEQ ID NO: 27 - DNA, 24 bp, Artificial Sequence
  Description of Artificial Sequence: Synthetic probe
agctctctcgacgcaggactcggc

SEQ ID NO: 28 - DNA, 21 bp, Artificial Sequence
  Description of Artificial Sequence: Synthetic primer
cactcccaacgaagacaagat

SEQ ID NO: 29 - DNA, 22 bp, Artificial Sequence
  Description of Artificial Sequence: Synthetic primer
gtctaaccagagagacccagta

SEQ ID NO: 30 - DNA, 24 bp, Artificial Sequence
  Description of Artificial Sequence: Synthetic probe
tttgtaaaccggtgcagctgcttt

SEQ ID NO: 31 - DNA, 21 bp, Artificial Sequence
  Description of Artificial Sequence: Synthetic primer
acctgaaagcgaaagggaaac

SEQ ID NO: 32 - DNA, 23 bp, Artificial Sequence
  Description of Artificial Sequence: Synthetic primer
cacccatctctctccttctagcc

SEQ ID NO: 33 - DNA, 24 bp, Artificial Sequence
  Description of Artificial Sequence: Synthetic probe
agctctctcgacgcaggactcggc

SEQ ID NO: 34 - DNA, 16777 bp, Artificial Sequence
  Description of Artificial Sequence: Synthetic polynucleotide
gtcgacggatcgggagatctcccgatcccctatggtgcactctcagtacaatctgctctgatgccgcatagttaagccagtatctgctccctgcttgtgtgttggaggtcgctgagtagtgcgcgagcaaaatttaagctacaacaaggcaaggcttgaccgacaattgcatgaagaatctgcttagggttaggcgttttgcgctgcttcgcgatgtacgggccagatatacgcgttgacattgattattgactagttattaatagtaatcaattacggggtcattagttcatagcccatatatggagttccgcgttacataacttacggtaaatggcccgcctggctgaccgcccaacgacccccgcccattgacgtcaataatgacgtatgttcccatagtaacgccaatagggactttccattgacgtcaatgggtggagtatttacggtaaactgcccacttggcagtacatcaagtgtatcatatgccaagtacgccccctattgacgtcaatgacggtaaatggcccgcctggcattatgcccagtacatgaccttatgggactttcctacttggcagtacatctacgtattagtcatcgctattaccatggtgatgcggttttggcagtacatcaatgggcgtggatagcggtttgactcacggggatttccaagtctccaccccattgacgtcaatgggagtttgttttggcaccaaaatcaacgggactttccaaaatgtcgtaacaactccgccccattgacgcaaatgggcggtaggcgtgtacggtgggaggtctatataagcagcgcgttttgcctgtactgggtctctctggttagaccagatctgagcctgggagctctctggctaactagggaacccactgcttaagcctcaataaagcttgccttgagtgcttcaagtagtgtgtgcccgtctgttgtgtgactctggtaactagagatccctcagacccttttagtcagtgtggaaaatctctagcagtggcgcccgaacagggacttgaaagcgaaagggaaaccagaggagctctctcgacgcaggactcggcttgctgaagcgcgcacggcaagaggcgaggggcggcgactggtgagtacgccaaaaattttgactagcggaggctagaaggagagagatgggtgcgagagcgtcagtattaagcgggggagaattagatcgcgatgggaaaaaattcggttaaggccagggggaaagaaaaaatataaattaaaacatatagtatgggcaagcagggagctagaacgattcgcagttaatcctggcctgttagaaacatcagaaggctgtagacaaatactgggacagctacaaccatcccttcagacaggatcagaagaacttagatcattatataatacagtagcaaccctctattgtgtgcatcaaaggatagagataaaagacaccaaggaagctttagacaagatagaggaagagcaaaacaaaagtaagaccaccgcacagcaagcggccgctgatcttcagacctggaggaggagatatgagggacaattggagaagtgaattatataaatataaagtagtaaaaattgaaccattaggagtagcacccaccaaggcaaagagaagagtggtgcagagagaaaaaagagcagtgggaataggagctttgttccttgggttcttgggagcagcaggaagcactatgggcgcagcgtcaatgacgctgacggtacaggccagacaattattgtctggtatagtgcagcagcagaacaatttgctgagggctattgaggcgcaacagcatctgttgcaactcacagtctggggcatcaagcagctccaggcaagaatcctggctgtggaaagatacctaaaggatcaacagctcctggggatttggggttgctctggaaaactcatttgcaccactgctgtgccttggaatgctagttggagtaataaatctctggaacagatttggaatcacacgacctggatggagtgggacagagaaattaacaattacacaagcttaatacactccttaattgaagaatcgcaaaaccagcaagaaaagaatgaacaagaattattggaattagataaatgggcaagtttgtggaattggtttaacataacaaattggctgtggtatataaaattattcataatgatagtaggaggcttggtaggtttaagaatagtttttgctgtactttctatagtgaatagagttaggcagggatattcaccattatcgtttcagacccacctcccaaccccgaggggacccgacaggcccgaaggaatagaagaagaaggtggagagagagacagagacagatccattcgattagtgaacggatcggcactgcgtgcgccaattctgcagacaaatggcagtattcatccacaattttaaaagaaaaggggggattggggggtacagtgcaggggaaagaatagtagacataatagcaacagacatacaaactaaagaattacaaaaacaaattacaaaaattcaaaattttcgggtttattacagggacagcagagatccagtttggttaattaagcattagttattaatagtaatcaattacggggtcattagttcatagcccatatatggagttccgcgttacataacttacggtaaatggcccgcctggttgaccgcccaacgacccccgcccattgacgtcaataatgacgtatgttcccatagtaacgccaatagggactttccattgacgtcaatgggtggagtatttacggtaaactgcccacttggtagtacatcaagtgtatcatacgccaagtacgccccctattgacgtcaatgacggtaaatggcccgcctggtattatgcccagtacatgaccttatgggactttcctacttggcagtacatctgcgtattagtcatcgctattaccatggtgatgcggttttggcagtacatcaatgggcgtggatagcggtttgactcacggggatttccaagtctccaccccattgacgtcaatgggagtttgttttggcaccaaaatcaacgggactttccaaaatgtcgtaacaactccgccccattgacgcaaatgggcggtaggcgtgtacggtgggaggtctatataagcagagctggtttagtgaaccgtcagatccgctagcattgtgtgcttttcgggccaccatgacgctgcggcttctggtggccgcgctctgcgccgggatcctggcagaggcgccccgagtgcgagcccagcacagggagagagtgacctgcacgcgcctttacgccgctgacattgtgttcttactggatggctcctcatccattggccgcagcaatttccgcgaggtccgcagctttctcgaagggctggtgctgcctttctctggagcagccagtgcacagggtgtgcgctttgccacagtgcagtacagcgatgacccacggacagagttcggcctggatgcacttggctctgggggtgatgtgatccgcgccatccgtgagcttagctacaaggggggcaacactcgcacaggggctgcaattctccatgtggctgaccatgtcttcctgccccagctggcccgacctggtgtccccaaggtctgcatcctgatcacagacgggaagtcccaggacctggtggacacagctgcccaaaggctgaaggggcagggggtcaagctatttgctgtggggatcaagaatgctgaccctgaggagctgaagcgagttgcctcacagcccaccagtgacttcttcttcttcgtcaatgacttcagcatcttgaggacactactgcccctcgtttcccggagagtgtgcacgactgctggtggcgtgcctgtgacccgacctccggatgactcgacctctgctccacgagacctggtgctgtctgagccaagcagccaatccttgagagtacagtggacagcggccagtggccctgtgactggctacaaggtccagtacactcctctgacggggctgggacagccactgccgagtgagcggcaggaggtgaacgtcccagctggtgagaccagtgtgcggctgcggggtctccggccactgaccgagtaccaagtgactgtgattgccctctacgccaacagcatcggggaggctgtgagcgggacagctcggaccactgccctagaagggccggaactgaccatccagaataccacagcccacagcctcctggtggcctggcggagtgtgccaggtgccactggctaccgtgtgacatggcgggtcctcagtggtgggcccacacagcagcaggagctgggccctgggcagggttcagtgttgctgcgtgacttggagcctggcacggactatgaggtgaccgtgagcaccctatttggccgcagtgtggggcccgccacttccctgatggctcgcactgacgcttctgttgagcagaccctgcgcccggtcatcctgggccccacatccatcctcctttcctggaacttggtgcctgaggcccgtggctaccggttggaatggcggcgtgagactggcttggagccaccgcagaaggtggtactgccctctgatgtgacccgctaccagttggatgggctgcagccgggcactgagtaccgcctcacactctacactctgctggagggccacgaggtggccacccctgcaaccgtggttcccactggaccagagctgcctgtgagccctgtaacagacctgcaagccaccgagctgcccgggcagcgggtgcgagtgtcctggagcccagtccctggtgccacccagtaccgcatcattgtgcgcagcacccagggggttgagcggaccctggtgcttcctgggagtcagacagcattcgacttggatgacgttcaggctgggcttagctacactgtgcgggtgtctgctcgagtgggtccccgtgagggcagtgccagtgtcctcactgtccgccgggagccggaaactccacttgctgttccagggctgcgggttgtggtgtcagatgcaacgcgagtgagggtggcctggggacccgtccctggagccagtggatttcggattagctggagcacaggcagtggtccggagtccagccagacactgcccccagactctactgccacagacatcacagggctgcagcctggaaccacctaccaggtggctgtgtcggtactgcgaggcagagaggagggccctgctgcagtcatcgtggctcgaacggacccactgggcccagtgaggacggtccatgtgactcaggccagcagctcatctgtcaccattacctggaccagggttcctggcgccacaggatacagggtttcctggcactcagcccacggcccagagaaatcccagttggtttctggggaggccacggtggctgagctggatggactggagccagatactgagtatacggtgcatgtgagggcccatgtggctggcgtggatgggccccctgcctctgtggttgtgaggactgcccctgagcctgtgggtcgtgtgtcgaggctgcagatcctcaatgcttccagcgacgttctacggatcacctgggtaggggtcactggagccacagcttacagactggcctggggccggagtgaaggcggccccatgaggcaccagatactcccaggaaacacagactctgcagagatccggggtctcgaaggtggagtcagctactcagtgcgagtgactgcacttgtcggggaccgcgagggcacacctgtctccattgttgtcactacgccgcctgaggctccgccagccctggggacgcttcacgtggtgcagcgcggggagcactcgctgaggctgcgctgggagccggtgcccagagcgcagggcttccttctgcactggcaacctgagggtggccaggaacagtcccgggtcctggggcccgagctcagcagctatcacctggacgggctggagccagcgacacagtaccgcgtgaggctgagtgtcctagggccggctggagaagggccctctgcagaggtgactgcgcgcactgagtcacctcgtgttccaagcattgaactacgtgtggtggacacctcgatcgactcggtgactttggcctggactccagtgtccagggcatccagctacatcctatcctggcggccactcagaggccctggccaggaagtgcctgggtccccgcagacacttccagggatctcaagctcccagcgggtgacagggctagagcctggcgtctcttacatcttctccctgacgcctgtcctggatggtgtgcggggtcctgaggcatctgtcacacagacgccagtgtgcccccgtggcctggcggatgtggtgttcctaccacatgccactcaagacaatgctcaccgtgcggaggctacgaggagggtcctggagcgtctggtgttggcacttgggcctcttgggccacaggcagttcaggttggcctgctgtcttacagtcatcggccctccccactgttcccactgaatggctcccatgaccttggcattatcttgcaaaggatccgtgacatgccctacatggacccaagtgggaacaacctgggcacagccgtggtcacagctcacagatacatgttggcaccagatgctcctgggcgccgccagcacgtaccaggggtgatggttctgctagtggatgaacccttgagaggtgacatattcagccccatccgtgaggcccaggcttctgggcttaatgtggtgatgttgggaatggctggagcggacccagagcagctgcgtcgcttggcgccgggtatggactctgtccagaccttcttcgccgtggatgatgggccaagcctggaccaggcagtcagtggtctggccacagccctgtgtcaggcatccttcactactcagccccggccagagccctgcccagtgtattgtccaaagggccagaagggggaacctggagagatgggcctgagaggacaagttgggcctcctggcgaccctggcctcccgggcaggaccggtgctcccggcccccaggggccccctggaagtgccactgccaagggcgagaggggcttccctggagcagatgggcgtccaggcagccctggccgcgccgggaatcctgggacccctggagcccctggcctaaagggctctccagggttgcctggccctcgtggggacccgggagagcgaggacctcgaggcccaaagggggagccgggggctcccggacaagtcatcggaggtgaaggacctgggcttcctgggcggaaaggggaccctggaccatcgggcccccctggacctcgtggaccactgggggacccaggaccccgtggccccccagggcttcctggaacagccatgaagggtgacaaaggcgatcgtggggagcggggtccccctggaccaggtgaaggtggcattgctcctggggagcctgggctgccgggtcttcccggaagccctggaccccaaggccccgttggcccccctggaaagaaaggagaaaaaggtgactctgaggatggagctccaggcctcccaggacaacctgggtctccgggtgagcagggcccacggggacctcctggagctattggccccaaaggtgaccggggctttccagggcccctgggtgaggctggagagaagggcgaacgtggacccccaggcccagcgggatcccgggggctgccaggggttgctggacgtcctggagccaagggtcctgaagggccaccaggacccactggccgccaaggagagaagggggagcctggtcgccctggggaccctgcagtggtgggacctgctgttgctggacccaaaggagaaaagggagatgtggggcccgctgggcccagaggagctaccggagtccaaggggaacggggcccacccggcttggttcttcctggagaccctggccccaagggagaccctggagaccggggtcccattggccttactggcagagcaggacccccaggtgactcagggcctcctggagagaagggagaccctgggcggcctggccccccaggacctgttggcccccgaggacgagatggtgaagttggagagaaaggtgacgagggtcctccgggtgacccgggtttgcctggaaaagcaggcgagcgtggccttcggggggcacctggagttcgggggcctgtgggtgaaaagggagaccagggagatcctggagaggatggacgaaatggcagccctggatcatctggacccaagggtgaccgtggggagccgggtcccccaggacccccgggacggctggtagacacaggacctggagccagagagaagggagagcctggggaccgcggacaagagggtcctcgagggcccaagggtgatcctggcctccctggagcccctggggaaaggggcattgaagggtttcggggacccccaggcccacagggggacccaggtgtccgaggcccagcaggagaaaagggtgaccggggtccccctgggctggatggccggagcggactggatgggaaaccaggagccgctgggccctctgggccgaatggtgctgcaggcaaagctggggacccagggagagacgggcttccaggcctccgtggagaacaaggcctccctggcccctctggtccccctggattaccgggaaagccaggcgaggatgggaaacctggcctgaatggaaaaaacggagaacctggggaccctggagaagacgggaggaagggagagaaaggagattcaggcgcctctgggagagaaggtcgtgatggccccaagggtgagcgtggagctcctggtatccttggaccccaggggcctccaggcctcccagggccagtgggccctcctggccagggttttcctggtgtcccaggaggcacgggccccaagggtgaccgtggggagactggatccaaaggggagcagggcctccctggagagcgtggcctgcgaggagagcctggaagtgtgccgaatgtggatcggttgctggaaactgctggcatcaaggcatctgccctgcgggagatcgtggagacctgggatgagagctctggtagcttcctgcctgtgcccgaacggcgtcgaggccccaagggggactcaggcgaacagggccccccaggcaaggagggccccatcggctttcctggagaacgcgggctgaagggcgaccgtggagaccctggccctcaggggccacctggtctggcccttggggagaggggcccccccgggccttccggccttgccggggagcctggaaagcctggtattcccgggctcccaggcagggctgggggtgtgggagaggcaggaaggccaggagagaggggagaacggggagagaaaggagaacgtggagaacagggcagagatggccctcctggactccctggaacccctgggccccccggaccccctggccccaaggtgtctgtggatgagccaggtcctggactctctggagaacagggaccccctggactcaagggtgctaagggggagccgggcagcaatggtgaccaaggtcccaaaggagacaggggtgtgccaggcatcaaaggagaccggggagagcctggaccgaggggtcaggacggcaacccgggtctaccaggagagcgtggtatggctgggcctgaagggaagccgggtctgcagggtccaagaggcccccctggcccagtgggtggtcatggagaccctggaccacctggtgccccgggtcttgctggccctgcaggaccccaaggaccttctggcctgaagggggagcctggagagacaggacctccaggacggggcctgactggacctactggagctgtgggacttcctggaccccccggcccttcaggccttgtgggtccacaggggtctccaggtttgcctggacaagtgggggagacagggaagccgggagccccaggtcgagatggtgccagtggaaaagatggagacagagggagccctggtgtgccagggtcaccaggtctgcctggccctgtcggacctaaaggagaacctggccccacgggggcccctggacaggctgtggtcgggctccctggagcaaagggagagaagggagcccctggaggccttgctggagacctggtgggtgagccgggagccaaaggtgaccgaggactgccagggccgcgaggcgagaagggtgaagctggccgtgcaggggagcccggagaccctggggaagatggtcagaaaggggctccaggacccaaaggtttcaagggtgacccaggagtcggggtcccgggctcccctgggcctcctggccctccaggtgtgaagggagatctgggcctccctggcctgcccggtgctcctggtgttgttgggttcccgggtcagacaggccctcgaggagagatgggtcagccaggccctagtggagagcggggtctggcaggccccccagggagagaaggaatcccaggacccctggggccacctggaccaccggggtcagtgggaccacctggggcctctggactcaaaggagacaagggagaccctggagtagggctgcctgggccccgaggcgagcgtggggagccaggcatccggggtgaagatggccgccccggccaggagggaccccgaggactcacggggccccctggcagcaggggagagcgtggggagaagggtgatgttgggagtgcaggactaaagggtgacaagggagactcagctgtgatcctggggcctccaggcccacggggtgccaagggggacatgggtgaacgagggcctcggggcttggatggtgacaaaggacctcggggagacaatggggaccctggtgacaagggcagcaagggagagcctggtgacaagggctcagccgggttgccaggactgcgtggactcctgggaccccagggtcaacctggtgcagcagggatccctggtgacccgggatccccaggaaaggatggagtgcctggtatccgaggagaaaaaggagatgttggcttcatgggtccccggggcctcaagggtgaacggggagtgaagggagcctgtggccttgatggagagaagggagacaagggagaagctggtcccccaggccgccccgggctggcaggacacaaaggagagatgggggagcctggtgtgccgggccagtcgggggcccctggcaaggagggcctgatcggtcccaagggtgaccgaggctttgacgggcagccaggccccaagggtgaccagggcgagaaaggggagcggggaaccccaggaattgggggcttcccaggccccagtggaaatgatggctctgctggtcccccagggccacctggcagtgttggtcccagaggccccgaaggacttcagggccagaagggtgagcgaggtccccccggagagagagtggtgggggctcctggggtccctggagctcctggcgagagaggggagcaggggcggccagggcctgccggtcctcgaggcgagaagggagaagctgcactgacggaggatgacatccggggctttgtgcgccaagagatgagtcagcactgtgcctgccagggccagttcatcgcatctggatcacgacccctccctagttatgctgcagacactgccggctcccagctccatgctgtgcctgtgctccgcgtctctcatgcagaggaggaagagcgggtaccccctgaggatgatgagtactctgaatactccgagtattctgtggaggagtaccaggaccctgaagctccttgggatagtgatgacccctgttccctgccactggatgagggctcctgcactgcctacaccctgcgctggtaccatcgggctgtgacaggcagcacagaggcctgtcacccttttgtctatggtggctgtggagggaatgccaaccgttttgggacccgtgaggcctgcgagcgccgctgcccaccccgggtggtccagagccaggggacaggtactgcccaggactgatcgataccgtcgacctcgagacctagaaaaacatggagcaatcacaagtagcaatacagcagctaccaatgctgattgtgcctggctagaagcacaagaggaggaggaggtgggttttccagtcacacctcaggtacctttaagaccaatgacttacaaggcagctgtagatcttagccactttttaaaagaaaaggggggactggaagggctaattcactcccaacgaagacaagatatccttgatctgtggatctaccacacacaaggctacttccctgattggcagaactacacaccagggccagggatcagatatccactgacctttggatggtgctacaagctagtaccagttgagcaagagaaggtagaagaagccaatgaaggagagaacacccgcttgttacaccctgtgagcctgcatgggatggatgacccggagagagaagtattagagtggaggtttgacagccgcctagcatttcatcacatggcccgagagctgcatccggactgtactgggtctctctggttagaccagatctgagcctgggagctctctggctaactagggaacccactgcttaagcctcaataaagcttgccttgagtgcttcaagtagtgtgtgcccgtctgttgtgtgactctggtaactagagatccctcagacccttttagtcagtgtggaaaatctctagcagggcccgtttaaacccgctgatcagcctcgactgtgccttctagttgccagccatctgttgtttgcccctcccccgtgccttccttgaccctggaaggtgccactcccactgtcctttcctaataaaatgaggaaattgcatcgcattgtctgagtaggtgtcattctattctggggggtggggtggggcaggacagcaagggggaggattgggaagacaatagcaggcatgctggggatgcggtgggctctatggcttctgaggcggaaagaaccagctggggctctagggggtatccccacgcgccctgtagcggcgcattaagcgcggcgggtgtggtggttacgcgcagcgtgaccgctacacttgccagcgccctagcgcccgctcctttcgctttcttcccttcctttctcgccacgttcgccggctttccccgtcaagctctaaatcgggggctccctttagggttccgatttagtgctttacggcacctcgaccccaaaaaacttgattagggtgatggttcacgtagtgggccatcgccctgatagacggtttttcgccctttgacgttggagtccacgttctttaatagtggactcttgttccaaactggaacaacactcaaccctatctcggtctattcttttgatttataagggattttgccgatttcggcctattggttaaaaaatgagctgatttaacaaaaatttaacgcgaattaattctgtggaatgtgtgtcagttagggtgtggaaagtccccaggctccccagcaggcagaagtatgcaaagcatgcatctcaattagtcagcaaccaggtgtggaaagtccccaggctccccagcaggcagaagtatgcaaagcatgcatctcaattagtcagcaaccatagtcccgcccctaactccgcccatcccgcccctaactccgcccagttccgcccattctccgccccatggctgactaattttttttatttatgcagaggccgaggccgcctctgcctctgagctattccagaagtagtgaggaggcttttttggaggcctaggcttttgcaaaaagctcccgggagcttgtatatccattttcggatctgatcagcacgtgttgacaattaatcatcggcatagtatatcggcatagtataatacgacaaggtgaggaactaaaccatggccaagttgaccagtgccgttccggtgctcaccgcgcgcgacgtcgccggagcggtcgagttctggaccgaccggctcgggttctcccgggacttcgtggaggacgacttcgccggtgtggtccgggacgacgtgaccctgttcatcagcgcggtccaggaccaggtggtgccggacaacaccctggcctgggtgtgggtgcgcggcctggacgagctgtacgccgagtggtcggaggtcgtgtccacgaacttccgggacgcctccgggccggccatgaccgagatcggcgagcagccgtgggggcgggagttcgccctgcgcgacccggccggcaactgcgtgcacttcgtggccgaggagcaggactgacacgtgctacgagatttcgattccaccgccgccttctatgaaaggttgggcttcggaatcgttttccgggacgccggctggatgatcctccagcgcggggatctcatgctggagttcttcgcccaccccaacttgtttattgcagcttataatggttacaaataaagcaatagcatcacaaatttcacaaataaagcatttttttcactgcattctagttgtggtttgtccaaactcatcaatgtatcttatcatgtctgtataccgtcgacctctagctagagcttggcgtaatcatggtcatagctgtttcctgtgtgaaattgttatccgctcacaattccacacaacatacgagccggaagcataaagtgtaaagcctggggtgcctaatgagtgagctaactcacattaattgcgttgcgctcactgcccgctttccagtcgggaaacctgtcgtgccagctgcattaatgaatcggccaacgcgcggggagaggcggtttgcgtattgggcgctcttccgcttcctcgctcactgactcgctgcgctcggtcgttcggctgcggcgagcggtatcagctcactcaaaggcggtaatacggttatccacagaatcaggggataacgcaggaaagaacatgtgagcaaaaggccagcaaaaggccaggaaccgtaaaaaggccgcgttgctggcgtttttccataggctccgcccccctgacgagcatcacaaaaatcgacgctcaagtcagaggtggcgaaacccgacaggactataaagataccaggcgtttccccctggaagctccctcgtgcgctctcctgttccgaccctgccgcttaccggatacctgtccgcctttctcccttcgggaagcgtggcgctttctcatagctcacgctgtaggtatctcagttcggtgtaggtcgttcgctccaagctgggctgtgtgcacgaaccccccgttcagcccgaccgctgcgccttatccggtaactatcgtcttgagtccaacccggtaagacacgacttatcgccactggcagcagccactggtaacaggattagcagagcgaggtatgtaggcggtgctacagagttcttgaagtggtggcctaactacggctacactagaagaacagtatttggtatctgcgctctgctgaagccagttaccttcggaaaaagagttggtagctcttgatccggcaaacaaaccaccgctggtagcggtggtttttttgtttgcaagcagcagattacgcgcagaaaaaaaggatctcaagaagatcctttgatcttttctacggggtctgacgctcagtggaacgaaaactcacgttaagggattttggtcatgagattatcaaaaaggatcttcacctagatccttttaaattaaaaatgaagttttaaatcaatctaaagtatatatgagtaaacttggtctgacagttaccaatgcttaatcagtgaggcacctatctcagcgatctgtctatttcgttcatccatagttgcctgactccccgtcgtgtagataactacgatacgggagggcttaccatctggccccagtgctgcaatgataccgcgagacccacgctcaccggctccagatttatcagcaataaaccagccagccggaagggccgagcgcagaagtggtcctgcaactttatccgcctccatccagtctattaattgttgccgggaagctagagtaagtagttcgccagttaatagtttgcgcaacgttgttgccattgctacaggcatcgtggtgtcacgctcgtcgtttggtatggcttcattcagctccggttcccaacgatcaaggcgagttacatgatcccccatgttgtgcaaaaaagcggttagctccttcggtcctccgatcgttgtcagaagtaagttggccgcagtgttatcactcatggttatggcagcactgcataattctcttactgtcatgccatccgtaagatgcttttctgtgactggtgagtactcaaccaagtcattctgagaatagtgtatgcggcgaccgagttgctcttgcccggcgtcaatacgggataataccgcgccacatagcagaactttaaaagtgctcatcattggaaaacgttcttcggggcgaaaactctcaaggatcttaccgctgttgagatccagttcgatgtaacccactcgtgcacccaactgatcttcagcatcttttactttcaccagcgtttctgggtgagcaaaaacaggaaggcaaaatgccgcaaaaaagggaataagggcgacacggaaatgttgaatactcatactcttcctttttcaatattattgaagcatttatcagggttattgtctcatgagcggatacatatttgaatgtatttagaaaaataaacaaataggggttccgcgcacatttccccgaaaagtgccacctgac